European Patent Application EP 4 570 971 A1, published June 18, 2025. Title: 次世代シーケンサー解析等のための断片化及びタグメント化方法. Applicant: 東洋紡株式会社. The sequence listing filed with the application follows.

SEQUENCE LISTING (17 sequences)

SEQ ID NO: 1 - DNA, 19 bp, synthetic construct
  source 1..19: mol_type = other DNA; note = transposon end sequence
agatgtgtataagagacag

SEQ ID NO: 2 - DNA, 19 bp, synthetic construct
  source 1..19: mol_type = other DNA; note = transposon end sequence
ctgtctcttatacacatct

SEQ ID NO: 3 - DNA, 49 bp, synthetic construct
  source 1..49: mol_type = other DNA; note = first adapter
tcgtcggcagcgtcctcgtgtgctacttgaagatgtgtataagagacag

SEQ ID NO: 4 - DNA, 19 bp, synthetic construct
  source 1..19: mol_type = other DNA; note = second adapter
ctgtctcttatacacatct

SEQ ID NO: 5 - DNA, 31 bp, synthetic construct
  source 1..31: mol_type = other DNA; note = additional oligo
tcaagtagcacacgagccgagcccacgagac

SEQ ID NO: 6 - DNA, 44 bp, synthetic construct
  source 1..44: mol_type = other DNA; note = first adapter
tcgtcggcagcgtcagctagctagcagatgtgtataagagacag

SEQ ID NO: 7 - DNA, 15 bp, synthetic construct
  source 1..15: mol_type = other DNA; note = second adapter
ctgtctcttatacac

SEQ ID NO: 8 - DNA, 30 bp, synthetic construct
  source 1..30: mol_type = other DNA; note = additional oligo
atctgctagctagctccgagcccacgagac

SEQ ID NO: 9 - DNA, 49 bp, synthetic construct
  source 1..49: mol_type = other DNA; note = first adapter
ctcgtgtgctacttgatcgtcggcagcgtcagatgtgtataagagacag

SEQ ID NO: 10 - DNA, 12 bp, synthetic construct
  source 1..12: mol_type = other DNA; note = second adapter
ctgtctcttata

SEQ ID NO: 11 - DNA, 38 bp, synthetic construct
  source 1..38: mol_type = other DNA; note = additional oligo
cacatctccgagcccacgagactcaagtagcacacgag

SEQ ID NO: 12 - DNA, 40 bp, synthetic construct
  source 1..40: mol_type = other DNA; note = read 1 primer
gcgtcctcgtgtgctacttgaagatgtgtataagagacag

SEQ ID NO: 13 - DNA, 40 bp, synthetic construct
  source 1..40: mol_type = other DNA; note = read 2 primer
ctcggctcgtgtgctacttgaagatgtgtataagagacag

SEQ ID NO: 14 - DNA, 31 bp, synthetic construct; identical to SEQ ID NO: 5
  source 1..31: mol_type = other DNA; note = index 1 read primer

SEQ ID NO: 15 - DNA, 39 bp, synthetic construct
  source 1..39: mol_type = other DNA; note = read 1 primer
ggcagcgtcagctagctagcagatgtgtataagagacag

SEQ ID NO: 16 - DNA, 40 bp, synthetic construct
  source 1..40: mol_type = other DNA; note = read 2 primer
gtgggctcggagctagctagcagatgtgtataagagacag

SEQ ID NO: 17 - DNA, 32 bp, synthetic construct
  source 1..32: mol_type = other DNA; note = index 1 read primer
acatctgctagctagctccgagcccacgagac